European Patent Application EP 4 410 808 A1, published August 7, 2024. Title: PEPTIDE HAVING ANTI-OBESITY ACTIVITY AND USES THEREOF. Applicant: CAREGEN CO., LTD. The sequence listing filed with the application follows.

SEQUENCE LISTING (17 sequences)

SEQ ID NO: 1 - protein, 10 aa, synthetic construct
  REGION 1..10: note = peptide
DYNMKWIHVY

SEQ ID NO: 2 - DNA, 20 bp, synthetic construct
  misc_feature 1..20: note = Perilipin1-F
  source 1..20: mol_type = other DNA
aaggatcctgcacctcacac

SEQ ID NO: 3 - DNA, 20 bp, synthetic construct
  misc_feature 1..20: note = Perilipin1-R
  source 1..20: mol_type = other DNA
cctctgctgaagggttatcg

SEQ ID NO: 4 - DNA, 17 bp, synthetic construct
  misc_feature 1..17: note = HSL-F
  source 1..17: mol_type = other DNA
ggacacacacacacctg

SEQ ID NO: 5 - DNA, 20 bp, synthetic construct
  misc_feature 1..20: note = HSL-R
  source 1..20: mol_type = other DNA
ccctttcgcagcaactttag

SEQ ID NO: 6 - DNA, 20 bp, synthetic construct
  misc_feature 1..20: note = ATGL-F
  source 1..20: mol_type = other DNA
tcgtggatgttggtggagct

SEQ ID NO: 7 - DNA, 19 bp, synthetic construct
  misc_feature 1..19: note = ATGL-R
  source 1..19: mol_type = other DNA
tgtggcctcattcctccta

SEQ ID NO: 8 - DNA, 20 bp, synthetic construct
  misc_feature 1..20: note = GAPDH-F
  source 1..20: mol_type = other DNA
gtgatggcatggactgtggt

SEQ ID NO: 9 - DNA, 20 bp, synthetic construct
  misc_feature 1..20: note = GAPDH-R
  source 1..20: mol_type = other DNA
ggagccaaaagggtcatcat

SEQ ID NO: 10 - DNA, 21 bp, synthetic construct
  misc_feature 1..21: note = PGCl alpha-F
  source 1..21: mol_type = other DNA
atgtgcagccaagactctgta

SEQ ID NO: 11 - DNA, 21 bp, synthetic construct
  misc_feature 1..21: note = PGCl alpha-R
  source 1..21: mol_type = other DNA
cgctacaccacttcaatccac

SEQ ID NO: 12 - DNA, 21 bp, synthetic construct
  misc_feature 1..21: note = Tbx1-F
  source 1..21: mol_type = other DNA
ctgtgggacgagttcaatcag

SEQ ID NO: 13 - DNA, 21 bp, synthetic construct
  misc_feature 1..21: note = Tbx1-R
  source 1..21: mol_type = other DNA
ttgtcatctacgggcacaaag

SEQ ID NO: 14 - DNA, 20 bp, synthetic construct
  misc_feature 1..20: note = FGF21-F
  source 1..20: mol_type = other DNA
cgtctgcctcagaaggactc

SEQ ID NO: 15 - DNA, 20 bp, synthetic construct
  misc_feature 1..20: note = FGF21-R
  source 1..20: mol_type = other DNA
tctaccatgctcagggggtc

SEQ ID NO: 16 - DNA, 20 bp, synthetic construct
  misc_feature 1..20: note = UCP1-F
  source 1..20: mol_type = other DNA
cctgcctctctcggaaacaa

SEQ ID NO: 17 - DNA, 20 bp, synthetic construct
  misc_feature 1..20: note = UCP1-R
  source 1..20: mol_type = other DNA
gtagcggggtttgatcccat